European Patent Specification EP 4 157 246 B1, published May 28, 2025. Title: Therapeutic combination for the treatment of breast cancer. Applicant: Università degli Studi di Genova IFOM - Fondazione Istituto FIRC di Oncologia Molecolare University of Southern California. The sequence listing filed with the application follows.

SEQUENCE LISTING (28 sequences)

SEQ ID NO: 1 - DNA, 24 bp, Unknown
  Primer
cgggaaatcgtgcgtgacattaag

SEQ ID NO: 2 - DNA, 24 bp, Unknown
  Primer
tgatctccttctgcatcctgtcgg

SEQ ID NO: 3 - DNA, 23 bp, Unknown
  Primer
tttggagcagagaggaggcaatg

SEQ ID NO: 4 - DNA, 24 bp, Unknown
  Primer
accacaattctgtctttcacgggg

SEQ ID NO: 5 - DNA, 20 bp, Unknown
  Primer
atgttttcctgtgccctgag

SEQ ID NO: 6 - DNA, 20 bp, Unknown
  Primer
atctgtggtgagggatgagg

SEQ ID NO: 7 - DNA, 22 bp, Unknown
  Primer
ctctctgagcttcaagcacctg

SEQ ID NO: 8 - DNA, 22 bp, Unknown
  Primer
cttgacggcaatcactgtctgc

SEQ ID NO: 9 - DNA, 22 bp, Unknown
  Primer
tgtgtcctggatgttgactgcc

SEQ ID NO: 10 - DNA, 23 bp, Unknown
  Primer
ctctatgtcgcaccactgatacc

SEQ ID NO: 11 - DNA, 20 bp, Unknown
  Primer
gcctctaagatgaaggagac

SEQ ID NO: 12 - DNA, 16 bp, Unknown
  Primer
ccatttgcagcagctc

SEQ ID NO: 13 - DNA, 18 bp, Unknown
  Primer
gcagagtcttttcctgac

SEQ ID NO: 14 - DNA, 18 bp, Unknown
  Primer
ttggtcatgctcactagg

SEQ ID NO: 15 - DNA, 19 bp, Unknown
  Primer
ggctaagtgaagatgacaa

SEQ ID NO: 16 - DNA, 20 bp, Unknown
  Primer
gttactccctttttgtctct

SEQ ID NO: 17 - DNA, 23 bp, Unknown
  Primer
tttggagcagagaggaggcaatg

SEQ ID NO: 18 - DNA, 24 bp, Unknown
  Primer
accacaattctgtctttcacgggg

SEQ ID NO: 19 - DNA, 20 bp, Unknown
  Primer
cttggtttctctgggaattg

SEQ ID NO: 20 - DNA, 20 bp, Unknown
  Primer
ttccaacagattaaaggtcc

SEQ ID NO: 21 - DNA, 20 bp, Unknown
  Primer
gatgtatgaaggctttggtc

SEQ ID NO: 22 - DNA, 20 bp, Unknown
  Primer
tgtgcacttttattggtctc

SEQ ID NO: 23 - DNA, 20 bp, Unknown
  Primer
cagagtccttttctgacatc

SEQ ID NO: 24 - DNA, 18 bp, Unknown
  Primer
gagaagcggccagtatag

SEQ ID NO: 25 - DNA, 20 bp, Unknown
  Primer
aacttgcaatcctcagtttg

SEQ ID NO: 26 - DNA, 22 bp, Unknown
  Primer
ctactttgatatcaccacacac

SEQ ID NO: 27 - DNA, 20 bp, Unknown
  Primer
ctcaagaagaagaatgtccc

SEQ ID NO: 28 - DNA, 20 bp, Unknown
  Primer
ctcttttaattctcaggccg